European Patent Application EP 4 218 784 A2, published August 2, 2023. Title: MACROCYCLIC MODULATORS OF DISEASE ASSOCIATED PROTEIN MISFOLDING AND AGGREGATION. Applicant: National Hellenic Research Foundation. Application EP. The sequence listing filed with the application follows.

SEQUENCE LISTING (255 sequences)

SEQ ID NO: 1 - protein, 5 aa, synthetic construct
  REGION 1..5: note = SOD1C5-1 peptide selected for its ability to rescue themisfolding and modulate the aggregation of SOD1
TASWW

SEQ ID NO: 2 - protein, 5 aa, synthetic construct
  REGION 1..5: note = SOD1C5-2 peptide selected for its ability to rescue themisfolding and modulate the aggregation of SOD1
TASFW

SEQ ID NO: 3 - protein, 5 aa, synthetic construct
  REGION 1..5: note = SOD1C5-3 peptide selected for its ability to rescue themisfolding and modulate the aggregation of SOD1
TSSFW

SEQ ID NO: 4 - protein, 5 aa, synthetic construct
  REGION 1..5: note = SOD1C5-4 peptide selected for its ability to rescue themisfolding and modulate the aggregation of SOD1
TWSVW

SEQ ID NO: 5 - protein, 5 aa, synthetic construct
  REGION 1..5: note = SOD1C5-5 peptide selected for its ability to rescue themisfolding and modulate the aggregation of SOD1
TASHW

SEQ ID NO: 6 - protein, 5 aa, synthetic construct
  REGION 1..5: note = SOD1C5-6 peptide selected for its ability to rescue themisfolding and modulate the aggregation of SOD1
TFSMW

SEQ ID NO: 7 - protein, 5 aa, synthetic construct
  REGION 1..5: note = SOD1C5-7 peptide selected for its ability to rescue themisfolding and modulate the aggregation of SOD1
TASMW

SEQ ID NO: 8 - protein, 5 aa, synthetic construct
  REGION 1..5: note = SOD1C5-9 peptide selected for its ability to rescue themisfolding and modulate the aggregation of SOD1
TVSFW

SEQ ID NO: 9 - protein, 5 aa, synthetic construct
  REGION 1..5: note = SOD1C5-11 peptide selected for its ability to rescue themisfolding and modulate the aggregation of SOD1
TLSFW

SEQ ID NO: 10 - protein, 5 aa, synthetic construct
  REGION 1..5: note = SOD1C5-13 peptide selected for its ability to rescue themisfolding and modulate the aggregation of SOD1
TASRW

SEQ ID NO: 11 - protein, 5 aa, synthetic construct
  REGION 1..5: note = SOD1C5-14 peptide selected for its ability to rescue themisfolding and modulate the aggregation of SOD1
TASSW

SEQ ID NO: 12 - protein, 5 aa, synthetic construct
  REGION 1..5: note = SOD1C5-18 peptide selected for its ability to rescue themisfolding and modulate the aggregation of SOD1
TASLW

SEQ ID NO: 13 - protein, 5 aa, synthetic construct
  REGION 1..5: note = SOD1C5-20 peptide selected for its ability to rescue themisfolding and modulate the aggregation of SOD1
TSSSW

SEQ ID NO: 14 - protein, 5 aa, synthetic construct
  REGION 1..5: note = SOD1C5-23 peptide selected for its ability to rescue themisfolding and modulate the aggregation of SOD1
TGSVW

SEQ ID NO: 15 - protein, 5 aa, synthetic construct
  REGION 1..5: note = SOD1C5-25 peptide selected for its ability to rescue themisfolding and modulate the aggregation of SOD1
TWSLW

SEQ ID NO: 16 - protein, 5 aa, synthetic construct
  REGION 1..5: note = SOD1C5-27 peptide selected for its ability to rescue themisfolding and modulate the aggregation of SOD1
TLSMW

SEQ ID NO: 17 - protein, 5 aa, synthetic construct
  REGION 1..5: note = SOD1C5-31 peptide selected for its ability to rescue themisfolding and modulate the aggregation of SOD1
TWSAW

SEQ ID NO: 18 - protein, 5 aa, synthetic construct
  REGION 1..5: note = SOD1C5-32 peptide selected for its ability to rescue themisfolding and modulate the aggregation of SOD1
TGSWW

SEQ ID NO: 19 - protein, 5 aa, synthetic construct
  REGION 1..5: note = SOD1C5-33 peptide selected for its ability to rescue themisfolding and modulate the aggregation of SOD1
TRSVW

SEQ ID NO: 20 - protein, 5 aa, synthetic construct
  REGION 1..5: note = SOD1C5-39 peptide selected for its ability to rescue themisfolding and modulate the aggregation of SOD1
TSSLW

SEQ ID NO: 21 - protein, 5 aa, synthetic construct
  REGION 1..5: note = SOD1C5-44 peptide selected for its ability to rescue themisfolding and modulate the aggregation of SOD1
TASTW

SEQ ID NO: 22 - protein, 5 aa, synthetic construct
  REGION 1..5: note = SOD1C5-46 peptide selected for its ability to rescue themisfolding and modulate the aggregation of SOD1
TSSVW

SEQ ID NO: 23 - protein, 5 aa, synthetic construct
  REGION 1..5: note = SOD1C5-53 peptide selected for its ability to rescue themisfolding and modulate the aggregation of SOD1
TTSWW

SEQ ID NO: 24 - protein, 5 aa, synthetic construct
  REGION 1..5: note = SOD1C5-65 peptide selected for its ability to rescue themisfolding and modulate the aggregation of SOD1
TASVW

SEQ ID NO: 25 - protein, 5 aa, synthetic construct
  REGION 1..5: note = SOD1C5-74 peptide selected for its ability to rescue themisfolding and modulate the aggregation of SOD1
TCSWW

SEQ ID NO: 26 - protein, 5 aa, synthetic construct
  REGION 1..5: note = SOD1C5-75 peptide selected for its ability to rescue themisfolding and modulate the aggregation of SOD1
TPSFW

SEQ ID NO: 27 - protein, 5 aa, synthetic construct
  REGION 1..5: note = SOD1C5-76 peptide selected for its ability to rescue themisfolding and modulate the aggregation of SOD1
TTSFW

SEQ ID NO: 28 - protein, 5 aa, synthetic construct
  REGION 1..5: note = SOD1C5-80 peptide selected for its ability to rescue themisfolding and modulate the aggregation of SOD1
TFSTW

SEQ ID NO: 29 - protein, 5 aa, synthetic construct
  REGION 1..5: note = SOD1C5-82 peptide selected for its ability to rescue themisfolding and modulate the aggregation of SOD1
TSSMW

SEQ ID NO: 30 - protein, 5 aa, synthetic construct
  REGION 1..5: note = SOD1C5-89 peptide selected for its ability to rescue themisfolding and modulate the aggregation of SOD1
TVSWW

SEQ ID NO: 31 - protein, 5 aa, synthetic construct
  REGION 1..5: note = SOD1C5-93 peptide selected for its ability to rescue themisfolding and modulate the aggregation of SOD1
TDSWW

SEQ ID NO: 32 - protein, 5 aa, synthetic construct
  REGION 1..5: note = SOD1C5-105 peptide selected for its ability to rescue themisfolding and modulate the aggregation of SOD1
TSSWW

SEQ ID NO: 33 - protein, 5 aa, synthetic construct
  REGION 1..5: note = SOD1C5-106 peptide selected for its ability to rescue themisfolding and modulate the aggregation of SOD1
TRSWW

SEQ ID NO: 34 - protein, 5 aa, synthetic construct
  REGION 1..5: note = SOD1C5-109 peptide selected for its ability to rescue themisfolding and modulate the aggregation of SOD1
TWSMW

SEQ ID NO: 35 - protein, 5 aa, synthetic construct
  REGION 1..5: note = SOD1C5-116 peptide selected for its ability to rescue themisfolding and modulate the aggregation of SOD1
TASGW

SEQ ID NO: 36 - protein, 5 aa, synthetic construct
  REGION 1..5: note = SOD1C5-130 peptide selected for its ability to rescue themisfolding and modulate the aggregation of SOD1
TPSWW

SEQ ID NO: 37 - protein, 5 aa, synthetic construct
  REGION 1..5: note = SOD1C5-135 peptide selected for its ability to rescue themisfolding and modulate the aggregation of SOD1
TRSFW

SEQ ID NO: 38 - protein, 5 aa, synthetic construct
  REGION 1..5: note = SOD1C5-140 peptide selected for its ability to rescue themisfolding and modulate the aggregation of SOD1
TSSYW

SEQ ID NO: 39 - protein, 5 aa, synthetic construct
  REGION 1..5: note = SOD1C5-143 peptide selected for its ability to rescue themisfolding and modulate the aggregation of SOD1
TLSVW

SEQ ID NO: 40 - protein, 5 aa, synthetic construct
  REGION 1..5: note = SOD1C5-148 peptide selected for its ability to rescue themisfolding and modulate the aggregation of SOD1
TYSWW

SEQ ID NO: 41 - protein, 5 aa, synthetic construct
  REGION 1..5: note = SOD1C5-160 peptide selected for its ability to rescue themisfolding and modulate the aggregation of SOD1
TFSVW

SEQ ID NO: 42 - protein, 5 aa, synthetic construct
  REGION 1..5: note = SOD1C5-164 peptide selected for its ability to rescue themisfolding and modulate the aggregation of SOD1
TCSVW

SEQ ID NO: 43 - protein, 5 aa, synthetic construct
  REGION 1..5: note = SOD1C5-167 peptide selected for its ability to rescue themisfolding and modulate the aggregation of SOD1
TVSSW

SEQ ID NO: 44 - protein, 5 aa, synthetic construct
  REGION 1..5: note = SOD1C5-168 peptide selected for its ability to rescue themisfolding and modulate the aggregation of SOD1
TRSHW

SEQ ID NO: 45 - protein, 5 aa, synthetic construct
  REGION 1..5: note = SOD1C5-182 peptide selected for its ability to rescue themisfolding and modulate the aggregation of SOD1
TGSAW

SEQ ID NO: 46 - protein, 5 aa, synthetic construct
  REGION 1..5: note = SOD1C5-188 peptide selected for its ability to rescue themisfolding and modulate the aggregation of SOD1
TASYW

SEQ ID NO: 47 - protein, 5 aa, synthetic construct
  REGION 1..5: note = C5-2 peptide selected for its ability to modulate theaggregation of the -amyloid peptide
TTYAR

SEQ ID NO: 48 - protein, 5 aa, synthetic construct
  REGION 1..5: note = C5-3 peptide selected for its ability to modulate theaggregation of the -amyloid peptide
TTVDR

SEQ ID NO: 49 - protein, 5 aa, synthetic construct
  REGION 1..5: note = C5-5 peptide selected for its ability to modulate theaggregation of the -amyloid peptide
TTTWR

SEQ ID NO: 50 - protein, 5 aa, synthetic construct
  REGION 1..5: note = C5-7 peptide selected for its ability to modulate theaggregation of the -amyloid peptide
TTLHR

SEQ ID NO: 51 - protein, 5 aa, synthetic construct
  REGION 1..5: note = C5-8 peptide selected for its ability to modulate theaggregation of the -amyloid peptide
TTFAR

SEQ ID NO: 52 - protein, 5 aa, synthetic construct
  REGION 1..5: note = C5-9 peptide selected for its ability to modulate theaggregation of the -amyloid peptide
TVLDR

SEQ ID NO: 53 - protein, 5 aa, synthetic construct
  REGION 1..5: note = C5-12 peptide selected for its ability to modulate theaggregation of the -amyloid peptide
TTWAR

SEQ ID NO: 54 - protein, 5 aa, synthetic construct
  REGION 1..5: note = C5-13 peptide selected for its ability to modulate theaggregation of the -amyloid peptide
TALDR

SEQ ID NO: 55 - protein, 5 aa, synthetic construct
  REGION 1..5: note = C5-15 peptide selected for its ability to modulate theaggregation of the -amyloid peptide
TANVR

SEQ ID NO: 56 - protein, 5 aa, synthetic construct
  REGION 1..5: note = C5-17 peptide selected for its ability to modulate theaggregation of the -amyloid peptide
TTTAR

SEQ ID NO: 57 - protein, 5 aa, synthetic construct
  REGION 1..5: note = C5-18 peptide selected for its ability to modulate theaggregation of the -amyloid peptide
TTIAR

SEQ ID NO: 58 - protein, 5 aa, synthetic construct
  REGION 1..5: note = C5-19 peptide selected for its ability to modulate theaggregation of the -amyloid peptide
TVWDR

SEQ ID NO: 59 - protein, 5 aa, synthetic construct
  REGION 1..5: note = C5-20 peptide selected for its ability to modulate theaggregation of the -amyloid peptide
TTISR

SEQ ID NO: 60 - protein, 5 aa, synthetic construct
  REGION 1..5: note = C5-21 peptide selected for its ability to modulate theaggregation of the -amyloid peptide
TTWCR

SEQ ID NO: 61 - protein, 5 aa, synthetic construct
  REGION 1..5: note = C5-22 peptide selected for its ability to modulate theaggregation of the -amyloid peptide
TVLWR

SEQ ID NO: 62 - protein, 5 aa, synthetic construct
  REGION 1..5: note = C5-25 peptide selected for its ability to modulate theaggregation of the -amyloid peptide
TTLAR

SEQ ID NO: 63 - protein, 5 aa, synthetic construct
  REGION 1..5: note = C5-26 peptide selected for its ability to modulate theaggregation of the -amyloid peptide
TAWCR

SEQ ID NO: 64 - protein, 5 aa, synthetic construct
  REGION 1..5: note = C5-27 peptide selected for its ability to modulate theaggregation of the -amyloid peptide
TTSAR

SEQ ID NO: 65 - protein, 5 aa, synthetic construct
  REGION 1..5: note = C5-29 peptide selected for its ability to modulate theaggregation of the -amyloid peptide
TTLER

SEQ ID NO: 66 - protein, 5 aa, synthetic construct
  REGION 1..5: note = C5-30 peptide selected for its ability to modulate theaggregation of the -amyloid peptide
TSTAR

SEQ ID NO: 67 - protein, 5 aa, synthetic construct
  REGION 1..5: note = C5-35 peptide selected for its ability to modulate theaggregation of the -amyloid peptide
TVRDR

SEQ ID NO: 68 - protein, 5 aa, synthetic construct
  REGION 1..5: note = C5-41 peptide selected for its ability to modulate theaggregation of the -amyloid peptide
TGWAR

SEQ ID NO: 69 - protein, 5 aa, synthetic construct
  REGION 1..5: note = C5-44 peptide selected for its ability to modulate theaggregation of the -amyloid peptide
TAWAR

SEQ ID NO: 70 - protein, 5 aa, synthetic construct
  REGION 1..5: note = C5-45 peptide selected for its ability to modulate theaggregation of the -amyloid peptide
TTWVR

SEQ ID NO: 71 - protein, 5 aa, synthetic construct
  REGION 1..5: note = C5-46 peptide selected for its ability to modulate theaggregation of the -amyloid peptide
TLLWR

SEQ ID NO: 72 - protein, 5 aa, synthetic construct
  REGION 1..5: note = C5-47 peptide selected for its ability to modulate theaggregation of the -amyloid peptide
TTIDR

SEQ ID NO: 73 - protein, 5 aa, synthetic construct
  REGION 1..5: note = C5-50 peptide selected for its ability to modulate theaggregation of the -amyloid peptide
TALAR

SEQ ID NO: 74 - protein, 5 aa, synthetic construct
  REGION 1..5: note = C5-51 peptide selected for its ability to modulate theaggregation of the -amyloid peptide
TSVDR

SEQ ID NO: 75 - protein, 5 aa, synthetic construct
  REGION 1..5: note = C5-53 peptide selected for its ability to modulate theaggregation of the -amyloid peptide
TTVWR

SEQ ID NO: 76 - protein, 5 aa, synthetic construct
  REGION 1..5: note = C5-66 peptide selected for its ability to modulate theaggregation of the -amyloid peptide
TTHWR

SEQ ID NO: 77 - protein, 5 aa, synthetic construct
  REGION 1..5: note = C5-67 peptide selected for its ability to modulate theaggregation of the -amyloid peptide
TARDR

SEQ ID NO: 78 - protein, 5 aa, synthetic construct
  REGION 1..5: note = C5-73 peptide selected for its ability to modulate theaggregation of the -amyloid peptide
TTRDR

SEQ ID NO: 79 - protein, 5 aa, synthetic construct
  REGION 1..5: note = C5-80 peptide selected for its ability to modulate theaggregation of the -amyloid peptide
TSVHR

SEQ ID NO: 80 - protein, 5 aa, synthetic construct
  REGION 1..5: note = C5-82 peptide selected for its ability to modulate theaggregation of the -amyloid peptide
TAVWR

SEQ ID NO: 81 - protein, 5 aa, synthetic construct
  REGION 1..5: note = C5-83 peptide selected for its ability to modulate theaggregation of the -amyloid peptide
TTGCR

SEQ ID NO: 82 - protein, 5 aa, synthetic construct
  REGION 1..5: note = C5-89 peptide selected for its ability to modulate theaggregation of the -amyloid peptide
TATDR

SEQ ID NO: 83 - protein, 5 aa, synthetic construct
  REGION 1..5: note = C5-94 peptide selected for its ability to modulate theaggregation of the -amyloid peptide
TVLFR

SEQ ID NO: 84 - protein, 5 aa, synthetic construct
  REGION 1..5: note = C5-102 peptide selected for its ability to modulate theaggregation of the -amyloid peptide
TTYNR

SEQ ID NO: 85 - protein, 5 aa, synthetic construct
  REGION 1..5: note = C5-105 peptide selected for its ability to modulate theaggregation of the -amyloid peptide
TVRWR

SEQ ID NO: 86 - protein, 5 aa, synthetic construct
  REGION 1..5: note = C5-116 peptide selected for its ability to modulate theaggregation of the -amyloid peptide
TAFDR

SEQ ID NO: 87 - protein, 5 aa, synthetic construct
  REGION 1..5: note = C5-117 peptide selected for its ability to modulate theaggregation of the -amyloid peptide
TTRCR

SEQ ID NO: 88 - protein, 5 aa, synthetic construct
  REGION 1..5: note = C5-118 peptide selected for its ability to modulate theaggregation of the -amyloid peptide
TTFWR

SEQ ID NO: 89 - protein, 5 aa, synthetic construct
  REGION 1..5: note = C5-121 peptide selected for its ability to modulate theaggregation of the -amyloid peptide
TIKDR

SEQ ID NO: 90 - protein, 5 aa, synthetic construct
  REGION 1..5: note = C5-123 peptide selected for its ability to modulate theaggregation of the -amyloid peptide
TTVHR

SEQ ID NO: 91 - protein, 5 aa, synthetic construct
  REGION 1..5: note = C5-126 peptide selected for its ability to modulate theaggregation of the -amyloid peptide
TTLLR

SEQ ID NO: 92 - protein, 5 aa, synthetic construct
  REGION 1..5: note = C5-129 peptide selected for its ability to modulate theaggregation of the -amyloid peptide
TTLFR

SEQ ID NO: 93 - protein, 5 aa, synthetic construct
  REGION 1..5: note = C5-130 peptide selected for its ability to modulate theaggregation of the -amyloid peptide
TAYHR

SEQ ID NO: 94 - protein, 5 aa, synthetic construct
  REGION 1..5: note = C5-136 peptide selected for its ability to modulate theaggregation of the -amyloid peptide
TALHR

SEQ ID NO: 95 - protein, 5 aa, synthetic construct
  REGION 1..5: note = C5-139 peptide selected for its ability to modulate theaggregation of the -amyloid peptide
TTSPR

SEQ ID NO: 96 - protein, 5 aa, synthetic construct
  REGION 1..5: note = C5-146 peptide selected for its ability to modulate theaggregation of the -amyloid peptide
TTWSR

SEQ ID NO: 97 - protein, 5 aa, synthetic construct
  REGION 1..5: note = C5-147 peptide selected for its ability to modulate theaggregation of the -amyloid peptide
TAMHR

SEQ ID NO: 98 - protein, 5 aa, synthetic construct
  REGION 1..5: note = C5-155 peptide selected for its ability to modulate theaggregation of the -amyloid peptide
TSLDR

SEQ ID NO: 99 - protein, 5 aa, synthetic construct
  REGION 1..5: note = C5-158 peptide selected for its ability to modulate theaggregation of the -amyloid peptide
TTGAR

SEQ ID NO: 100 - protein, 5 aa, synthetic construct
  REGION 1..5: note = C5-162 peptide selected for its ability to modulate theaggregation of the -amyloid peptide
TSVWR

SEQ ID NO: 101 - protein, 5 aa, synthetic construct
  REGION 1..5: note = C5-173 peptide selected for its ability to modulate theaggregation of the -amyloid peptide
TTHAR

SEQ ID NO: 102 - protein, 5 aa, synthetic construct
  REGION 1..5: note = C5-176 peptide selected for its ability to modulate theaggregation of the -amyloid peptide
TAGWR

SEQ ID NO: 103 - protein, 5 aa, synthetic construct
  REGION 1..5: note = C5-177 peptide selected for its ability to modulate theaggregation of the -amyloid peptide
TATAR

SEQ ID NO: 104 - protein, 5 aa, synthetic construct
  REGION 1..5: note = C5-184 peptide selected for its ability to modulate theaggregation of the -amyloid peptide
TVLAR

SEQ ID NO: 105 - protein, 5 aa, synthetic construct
  REGION 1..5: note = C5-185 peptide selected for its ability to modulate theaggregation of the -amyloid peptide
TTFNR

SEQ ID NO: 106 - protein, 5 aa, synthetic construct
  REGION 1..5: note = C5-188 peptide selected for its ability to modulate theaggregation of the -amyloid peptide
TGMRR

SEQ ID NO: 107 - protein, 5 aa, synthetic construct
  REGION 1..5: note = C5-189 peptide selected for its ability to modulate theaggregation of the -amyloid peptide
TTVAR

SEQ ID NO: 108 - protein, 5 aa, synthetic construct
  REGION 1..5: note = AC5-190 peptide selected for its ability to modulate theaggregation of the -amyloid peptide
TLCLR

SEQ ID NO: 109 - protein, 5 aa, synthetic construct
  REGION 1..5: note = C5-192 peptide selected for its ability to modulate theaggregation of the -amyloid peptide
TGLAR

SEQ ID NO: 110 - protein, 5 aa, synthetic construct
  REGION 1..5: note = C5-198 peptide selected for its ability to modulate theaggregation of the -amyloid peptide
TSWCR

SEQ ID NO: 111 - protein, 5 aa, synthetic construct
  REGION 1..5: note = C5-209 peptide selected for its ability to modulate theaggregation of the -amyloid peptide
TTRAR

SEQ ID NO: 112 - protein, 5 aa, synthetic construct
  REGION 1..5: note = C5-215 peptide selected for its ability to modulate theaggregation of the -amyloid peptide
TTPWR

SEQ ID NO: 113 - protein, 5 aa, synthetic construct
  REGION 1..5: note = C5-218 peptide selected for its ability to modulate theaggregation of the -amyloid peptide
TVLHR

SEQ ID NO: 114 - protein, 5 aa, synthetic construct
  REGION 1..5: note = C5-223 peptide selected for its ability to modulate theaggregation of the -amyloid peptide
TGLDR

SEQ ID NO: 115 - protein, 5 aa, synthetic construct
  REGION 1..5: note = C5-230 peptide selected for its ability to modulate theaggregation of the -amyloid peptide
TTSDR

SEQ ID NO: 116 - protein, 5 aa, synthetic construct
  REGION 1..5: note = C5-239 peptide selected for its ability to modulate theaggregation of the -amyloid peptide
TTMHR

SEQ ID NO: 117 - protein, 5 aa, synthetic construct
  REGION 1..5: note = C5-242 peptide selected for its ability to modulate theaggregation of the -amyloid peptide
TTSTR

SEQ ID NO: 118 - protein, 5 aa, synthetic construct
  REGION 1..5: note = C5-244 peptide selected for its ability to modulate theaggregation of the -amyloid peptide
TTRVR

SEQ ID NO: 119 - protein, 5 aa, synthetic construct
  REGION 1..5: note = C5-245 peptide selected for its ability to modulate theaggregation of the -amyloid peptide
TTRFR

SEQ ID NO: 120 - protein, 5 aa, synthetic construct
  REGION 1..5: note = C5-248 peptide selected for its ability to modulate theaggregation of the -amyloid peptide
TTTHR

SEQ ID NO: 121 - protein, 5 aa, synthetic construct
  REGION 1..5: note = C5-250 peptide selected for its ability to modulate theaggregation of the -amyloid peptide
THAWR

SEQ ID NO: 122 - protein, 5 aa, synthetic construct
  REGION 1..5: note = C5-252 peptide selected for its ability to modulate theaggregation of the -amyloid peptide
TVIWR

SEQ ID NO: 123 - protein, 5 aa, synthetic construct
  REGION 1..5: note = C5-253 peptide selected for its ability to modulate theaggregation of the -amyloid peptide
TTWFR

SEQ ID NO: 124 - protein, 5 aa, synthetic construct
  REGION 1..5: note = C5-255 peptide selected for its ability to modulate theaggregation of the -amyloid peptide
TTSRR

SEQ ID NO: 125 - protein, 5 aa, synthetic construct
  REGION 1..5: note = C5-258 peptide selected for its ability to modulate theaggregation of the -amyloid peptide
TTSCR

SEQ ID NO: 126 - protein, 5 aa, synthetic construct
  REGION 1..5: note = C5-260 peptide selected for its ability to modulate theaggregation of the -amyloid peptide
TTWTR

SEQ ID NO: 127 - protein, 5 aa, synthetic construct
  REGION 1..5: note = C5-262 peptide selected for its ability to modulate theaggregation of the -amyloid peptide
TTSSR

SEQ ID NO: 128 - protein, 5 aa, synthetic construct
  REGION 1..5: note = C5-263 peptide selected for its ability to modulate theaggregation of the -amyloid peptide
THLAR

SEQ ID NO: 129 - protein, 5 aa, synthetic construct
  REGION 1..5: note = C5-264 peptide selected for its ability to modulate theaggregation of the -amyloid peptide
TSGAR

SEQ ID NO: 130 - protein, 5 aa, synthetic construct
  REGION 1..5: note = C5-266 peptide selected for its ability to modulate theaggregation of the -amyloid peptide
TTLRR

SEQ ID NO: 131 - protein, 5 aa, synthetic construct
  REGION 1..5: note = C5-270 peptide selected for its ability to modulate theaggregation of the -amyloid peptide
TATWR

SEQ ID NO: 132 - protein, 5 aa, synthetic construct
  REGION 1..5: note = C5-272 peptide selected for its ability to modulate theaggregation of the -amyloid peptide
TCMWR

SEQ ID NO: 133 - protein, 5 aa, synthetic construct
  REGION 1..5: note = C5-275 peptide selected for its ability to modulate theaggregation of the -amyloid peptide
TAHVR

SEQ ID NO: 134 - protein, 5 aa, synthetic construct
  REGION 1..5: note = C5-276 peptide selected for its ability to modulate theaggregation of the -amyloid peptide
TSWAR

SEQ ID NO: 135 - protein, 5 aa, synthetic construct
  REGION 1..5: note = C5-278 peptide selected for its ability to modulate theaggregation of the -amyloid peptide
TTWLR

SEQ ID NO: 136 - protein, 5 aa, synthetic construct
  REGION 1..5: note = C5-291 peptide selected for its ability to modulate theaggregation of the -amyloid peptide
TTLDR

SEQ ID NO: 137 - protein, 5 aa, synthetic construct
  REGION 1..5: note = C5-294 peptide selected for its ability to modulate theaggregation of the -amyloid peptide
TTPHR

SEQ ID NO: 138 - protein, 5 aa, synthetic construct
  REGION 1..5: note = C5-298 peptide selected for its ability to modulate theaggregation of the -amyloid peptide
TTRGR

SEQ ID NO: 139 - protein, 5 aa, synthetic construct
  REGION 1..5: note = C5-299 peptide selected for its ability to modulate theaggregation of the -amyloid peptide
TTVGR

SEQ ID NO: 140 - protein, 5 aa, synthetic construct
  REGION 1..5: note = C5-301 peptide selected for its ability to modulate theaggregation of the -amyloid peptide
TTTRR

SEQ ID NO: 141 - protein, 5 aa, synthetic construct
  REGION 1..5: note = C5-304 peptide selected for its ability to modulate theaggregation of the -amyloid peptide
TSINR

SEQ ID NO: 142 - protein, 5 aa, synthetic construct
  REGION 1..5: note = C5-305 peptide selected for its ability to modulate theaggregation of the -amyloid peptide
TTADR

SEQ ID NO: 143 - protein, 5 aa, synthetic construct
  REGION 1..5: note = C5-315 peptide selected for its ability to modulate theaggregation of the -amyloid peptide
TTSER

SEQ ID NO: 144 - protein, 5 aa, synthetic construct
  REGION 1..5: note = C5-316 peptide selected for its ability to modulate theaggregation of the -amyloid peptide
TTCAR

SEQ ID NO: 145 - protein, 5 aa, synthetic construct
  REGION 1..5: note = C5-317 peptide selected for its ability to modulate theaggregation of the -amyloid peptide
TTAWR

SEQ ID NO: 146 - protein, 5 aa, synthetic construct
  REGION 1..5: note = C5-320 peptide selected for its ability to modulate theaggregation of the -amyloid peptide
TTVER

SEQ ID NO: 147 - protein, 5 aa, synthetic construct
  REGION 1..5: note = C5-321 peptide selected for its ability to modulate theaggregation of the -amyloid peptide
TTTFR

SEQ ID NO: 148 - protein, 5 aa, synthetic construct
  REGION 1..5: note = C5-323 peptide selected for its ability to modulate theaggregation of the -amyloid peptide
TAVDR

SEQ ID NO: 149 - protein, 5 aa, synthetic construct
  REGION 1..5: note = C5-325 peptide selected for its ability to modulate theaggregation of the -amyloid peptide
TVWIR

SEQ ID NO: 150 - protein, 5 aa, synthetic construct
  REGION 1..5: note = C5-329 peptide selected for its ability to modulate theaggregation of the -amyloid peptide
TTVRR

SEQ ID NO: 151 - protein, 5 aa, synthetic construct
  REGION 1..5: note = C5-333 peptide selected for its ability to modulate theaggregation of the -amyloid peptide
THVRR

SEQ ID NO: 152 - protein, 5 aa, synthetic construct
  REGION 1..5: note = C5-343 peptide selected for its ability to modulate theaggregation of the -amyloid peptide
TNLDR

SEQ ID NO: 153 - protein, 5 aa, synthetic construct
  REGION 1..5: note = C5-344 peptide selected for its ability to modulate theaggregation of the -amyloid peptide
TTPGR

SEQ ID NO: 154 - protein, 5 aa, synthetic construct
  REGION 1..5: note = C5-348 peptide selected for its ability to modulate theaggregation of the -amyloid peptide
TTLTR

SEQ ID NO: 155 - protein, 5 aa, synthetic construct
  REGION 1..5: note = C5-355 peptide selected for its ability to modulate theaggregation of the -amyloid peptide
TATVR

SEQ ID NO: 156 - protein, 5 aa, synthetic construct
  REGION 1..5: note = C5-359 peptide selected for its ability to modulate theaggregation of the -amyloid peptide
TAMWR

SEQ ID NO: 157 - protein, 5 aa, synthetic construct
  REGION 1..5: note = C5-361 peptide selected for its ability to modulate theaggregation of the -amyloid peptide
TTKWR

SEQ ID NO: 158 - protein, 5 aa, synthetic construct
  REGION 1..5: note = C5-362 peptide selected for its ability to modulate theaggregation of the -amyloid peptide
TTWDR

SEQ ID NO: 159 - protein, 5 aa, synthetic construct
  REGION 1..5: note = C5-364 peptide selected for its ability to modulate theaggregation of the -amyloid peptide
TTMAR

SEQ ID NO: 160 - protein, 5 aa, synthetic construct
  REGION 1..5: note = C5-365 peptide selected for its ability to modulate theaggregation of the -amyloid peptide
TTGGR

SEQ ID NO: 161 - protein, 5 aa, synthetic construct
  REGION 1..5: note = C5-366 peptide selected for its ability to modulate theaggregation of the -amyloid peptide
TTMVR

SEQ ID NO: 162 - protein, 5 aa, synthetic construct
  REGION 1..5: note = C5-375 peptide selected for its ability to modulate theaggregation of the -amyloid peptide
TNLAR

SEQ ID NO: 163 - protein, 5 aa, synthetic construct
  REGION 1..5: note = C5-376 peptide selected for its ability to modulate theaggregation of the -amyloid peptide
TIRDR

SEQ ID NO: 164 - protein, 5 aa, synthetic construct
  REGION 1..5: note = C5-378 peptide selected for its ability to modulate theaggregation of the -amyloid peptide
TTTGR

SEQ ID NO: 165 - protein, 5 aa, synthetic construct
  REGION 1..5: note = C5-379 peptide selected for its ability to modulate theaggregation of the -amyloid peptide
TRLGR

SEQ ID NO: 166 - protein, 5 aa, synthetic construct
  REGION 1..5: note = C5-381 peptide selected for its ability to modulate theaggregation of the -amyloid peptide
TTHTR

SEQ ID NO: 167 - protein, 5 aa, synthetic construct
  REGION 1..5: note = C5-382 peptide selected for its ability to modulate theaggregation of the -amyloid peptide
TTITR

SEQ ID NO: 168 - protein, 5 aa, synthetic construct
  REGION 1..5: note = C5-384 peptide selected for its ability to modulate theaggregation of the -amyloid peptide
TTYTR

SEQ ID NO: 169 - protein, 5 aa, synthetic construct
  REGION 1..5: note = C5-385 peptide selected for its ability to modulate theaggregation of the -amyloid peptide
TTLYR

SEQ ID NO: 170 - protein, 5 aa, synthetic construct
  REGION 1..5: note = C5-389 peptide selected for its ability to modulate theaggregation of the -amyloid peptide
THLDR

SEQ ID NO: 171 - protein, 5 aa, synthetic construct
  REGION 1..5: note = C5-391 peptide selected for its ability to modulate theaggregation of the -amyloid peptide
TLLIR

SEQ ID NO: 172 - protein, 5 aa, synthetic construct
  REGION 1..5: note = C5-392 peptide selected for its ability to modulate theaggregation of the -amyloid peptide
TTCDR

SEQ ID NO: 173 - protein, 5 aa, synthetic construct
  REGION 1..5: note = C5-393 peptide selected for its ability to modulate theaggregation of the -amyloid peptide
TTGRR

SEQ ID NO: 174 - protein, 5 aa, synthetic construct
  REGION 1..5: note = C5-394 peptide selected for its ability to modulate theaggregation of the -amyloid peptide
TTVSR

SEQ ID NO: 175 - protein, 5 aa, synthetic construct
  REGION 1..5: note = C5-395 peptide selected for its ability to modulate theaggregation of the -amyloid peptide
TTQHR

SEQ ID NO: 176 - protein, 5 aa, synthetic construct
  REGION 1..5: note = C5-396 peptide selected for its ability to modulate theaggregation of the -amyloid peptide
TTTPR

SEQ ID NO: 177 - protein, 5 aa, synthetic construct
  REGION 1..5: note = C5-399 peptide selected for its ability to modulate theaggregation of the -amyloid peptide
TAFAR

SEQ ID NO: 178 - protein, 5 aa, synthetic construct
  REGION 1..5: note = C5-405 peptide selected for its ability to modulate theaggregation of the -amyloid peptide
TTSHR

SEQ ID NO: 179 - protein, 5 aa, synthetic construct
  REGION 1..5: note = C5-410 peptide selected for its ability to modulate theaggregation of the -amyloid peptide
TVLGR

SEQ ID NO: 180 - protein, 5 aa, synthetic construct
  REGION 1..5: note = C5-411 peptide selected for its ability to modulate theaggregation of the -amyloid peptide
TTQRR

SEQ ID NO: 181 - protein, 5 aa, synthetic construct
  REGION 1..5: note = C5-413 peptide selected for its ability to modulate theaggregation of the -amyloid peptide
TSHAR

SEQ ID NO: 182 - protein, 5 aa, synthetic construct
  REGION 1..5: note = C5-415 peptide selected for its ability to modulate theaggregation of the -amyloid peptide
TTTCR

SEQ ID NO: 183 - protein, 5 aa, synthetic construct
  REGION 1..5: note = C5-422 peptide selected for its ability to modulate theaggregation of the -amyloid peptide
TAWRR

SEQ ID NO: 184 - protein, 5 aa, synthetic construct
  REGION 1..5: note = C5-428 peptide selected for its ability to modulate theaggregation of the -amyloid peptide
TTCGR

SEQ ID NO: 185 - protein, 5 aa, synthetic construct
  REGION 1..5: note = C5-434 peptide selected for its ability to modulate theaggregation of the -amyloid peptide
TTSGR

SEQ ID NO: 186 - protein, 5 aa, synthetic construct
  REGION 1..5: note = C5-438 peptide selected for its ability to modulate theaggregation of the -amyloid peptide
TTTSR

SEQ ID NO: 187 - protein, 5 aa, synthetic construct
  REGION 1..5: note = C5-440 peptide selected for its ability to modulate theaggregation of the -amyloid peptide
TATGR

SEQ ID NO: 188 - protein, 5 aa, synthetic construct
  REGION 1..5: note = C5-441 peptide selected for its ability to modulate theaggregation of the -amyloid peptide
TAWDR

SEQ ID NO: 189 - protein, 5 aa, synthetic construct
  REGION 1..5: note = C5-443 peptide selected for its ability to modulate theaggregation of the -amyloid peptide
TTHHR

SEQ ID NO: 190 - protein, 5 aa, synthetic construct
  REGION 1..5: note = C5-448 peptide selected for its ability to modulate theaggregation of the -amyloid peptide
TAYAR

SEQ ID NO: 191 - protein, 5 aa, synthetic construct
  REGION 1..5: note = C5-449 peptide selected for its ability to modulate theaggregation of the -amyloid peptide
TANAR

SEQ ID NO: 192 - protein, 5 aa, synthetic construct
  REGION 1..5: note = C5-450 peptide selected for its ability to modulate theaggregation of the -amyloid peptide
TRDVR

SEQ ID NO: 193 - protein, 5 aa, synthetic construct
  REGION 1..5: note = C5-452 peptide selected for its ability to modulate theaggregation of the -amyloid peptide
THVDR

SEQ ID NO: 194 - protein, 5 aa, synthetic construct
  REGION 1..5: note = C5-453 peptide selected for its ability to modulate theaggregation of the -amyloid peptide
TLFWR

SEQ ID NO: 195 - protein, 5 aa, synthetic construct
  REGION 1..5: note = C5-459 peptide selected for its ability to modulate theaggregation of the -amyloid peptide
TTAAR

SEQ ID NO: 196 - protein, 5 aa, synthetic construct
  REGION 1..5: note = C5-463 peptide selected for its ability to modulate theaggregation of the -amyloid peptide
TVVDR

SEQ ID NO: 197 - protein, 5 aa, synthetic construct
  REGION 1..5: note = C5-464 peptide selected for its ability to modulate theaggregation of the -amyloid peptide
TTPAR

SEQ ID NO: 198 - protein, 5 aa, synthetic construct
  REGION 1..5: note = C5-469 peptide selected for its ability to modulate theaggregation of the -amyloid peptide
TTIGR

SEQ ID NO: 199 - protein, 5 aa, synthetic construct
  REGION 1..5: note = C5-472 peptide selected for its ability to modulate theaggregation of the -amyloid peptide
TMYAR

SEQ ID NO: 200 - protein, 5 aa, synthetic construct
  REGION 1..5: note = C5-473 peptide selected for its ability to modulate theaggregation of the -amyloid peptide
THVAR

SEQ ID NO: 201 - protein, 5 aa, synthetic construct
  REGION 1..5: note = C5-474 peptide selected for its ability to modulate theaggregation of the -amyloid peptide
TTWPR

SEQ ID NO: 202 - protein, 5 aa, synthetic construct
  REGION 1..5: note = C5-475 peptide selected for its ability to modulate theaggregation of the -amyloid peptide
TTGDR

SEQ ID NO: 203 - protein, 5 aa, synthetic construct
  REGION 1..5: note = C5-479 peptide selected for its ability to modulate theaggregation of the -amyloid peptide
TTTVR

SEQ ID NO: 204 - protein, 5 aa, synthetic construct
  REGION 1..5: note = C5-481 peptide selected for its ability to modulate theaggregation of the -amyloid peptide
TVFGR

SEQ ID NO: 205 - protein, 5 aa, synthetic construct
  REGION 1..5: note = C5-483 peptide selected for its ability to modulate theaggregation of the -amyloid peptide
TRVGR

SEQ ID NO: 206 - protein, 5 aa, synthetic construct
  REGION 1..5: note = C5-34 peptide selected for its ability to modulate theaggregation of the -amyloid peptide
SASPT

SEQ ID NO: 207 - protein, 5 aa, synthetic construct
  REGION 1..5: note = C5-216 peptide selected for its ability to modulate theaggregation of the -amyloid peptide
SICPT

SEQ ID NO: 208 - protein, 5 aa, synthetic construct
  REGION 1..5: note = C5-380 peptide selected for its ability to modulate theaggregation of the -amyloid peptide
SITPT

SEQ ID NO: 209 - protein, 5 aa, synthetic construct
  REGION 1..5: note = C5-387 peptide selected for its ability to modulate theaggregation of the -amyloid peptide
SHSPT

SEQ ID NO: 210 - protein, 4 aa, synthetic construct
  REGION 1..4: note = C4-9 peptide selected for its ability to modulate theaggregation of the -amyloid peptide
TTCR

SEQ ID NO: 211 - protein, 4 aa, synthetic construct
  REGION 1..4: note = C4-11 peptide selected for its ability to modulate theaggregation of the -amyloid peptide
TTRR

SEQ ID NO: 212 - protein, 4 aa, synthetic construct
  REGION 1..4: note = C4-31 peptide selected for its ability to modulate theaggregation of the -amyloid peptide
TTSR

SEQ ID NO: 213 - protein, 4 aa, synthetic construct
  REGION 1..4: note = C4-34 peptide selected for its ability to modulate theaggregation of the -amyloid peptide
TRGR

SEQ ID NO: 214 - protein, 4 aa, synthetic construct
  REGION 1..4: note = C4-35 peptide selected for its ability to modulate theaggregation of the -amyloid peptide
TTGR

SEQ ID NO: 215 - protein, 4 aa, synthetic construct
  REGION 1..4: note = C4-41 peptide selected for its ability to modulate theaggregation of the -amyloid peptide
TRRR

SEQ ID NO: 216 - protein, 4 aa, synthetic construct
  REGION 1..4: note = AC4B-9 peptide selected for its ability to modulate theaggregation of the -amyloid peptide
TDQR

SEQ ID NO: 217 - protein, 4 aa, synthetic construct
  REGION 1..4: note = AC4B-41 peptide selected for its ability to modulate theaggregation of the -amyloid peptide
TLIR

SEQ ID NO: 218 - protein, 4 aa, synthetic construct
  REGION 1..4: note = AC4B-80 peptide selected for its ability to modulate theaggregation of the -amyloid peptide
TLWR

SEQ ID NO: 219 - protein, 4 aa, synthetic construct
  REGION 1..4: note = AC4B-86 peptide selected for its ability to modulate theaggregation of the -amyloid peptide
TLGR

SEQ ID NO: 220 - protein, 4 aa, synthetic construct
  REGION 1..4: note = C5(2) peptide selected for its ability to modulate theaggregation of the -amyloid peptide
TFDR

SEQ ID NO: 221 - protein, 4 aa, synthetic construct
  REGION 1..4: note = C5(D4) peptide selected for its ability to modulate theaggregation of the -amyloid peptide
TAFR

SEQ ID NO: 222 - protein, 6 aa, synthetic construct
  REGION 1..6: note = AC6-1 peptide selected for its ability to modulate theaggregation of the -amyloid peptide
TPVWFD

SEQ ID NO: 223 - protein, 6 aa, synthetic construct
  REGION 1..6: note = AC6-2 peptide selected for its ability to modulate theaggregation of the -amyloid peptide
TPAWFD

SEQ ID NO: 224 - protein, 6 aa, synthetic construct
  REGION 1..6: note = AC6-4 peptide selected for its ability to modulate theaggregation of the -amyloid peptide
TLEFFD

SEQ ID NO: 225 - protein, 6 aa, synthetic construct
  REGION 1..6: note = AC6-6 peptide selected for its ability to modulate theaggregation of the -amyloid peptide
TVTWFD

SEQ ID NO: 226 - protein, 6 aa, synthetic construct
  REGION 1..6: note = AC6-8 peptide selected for its ability to modulate theaggregation of the -amyloid peptide
TLLIRW

SEQ ID NO: 227 - protein, 6 aa, synthetic construct
  REGION 1..6: note = AC6-10 peptide selected for its ability to modulate theaggregation of the -amyloid peptide
TLKWLN

SEQ ID NO: 228 - protein, 6 aa, synthetic construct
  REGION 1..6: note = AC6-21 peptide selected for its ability to modulate theaggregation of the -amyloid peptide
TKEYFD

SEQ ID NO: 229 - protein, 6 aa, synthetic construct
  REGION 1..6: note = AC6-26 peptide selected for its ability to modulate theaggregation of the -amyloid peptide
TLHWFE

SEQ ID NO: 230 - protein, 6 aa, synthetic construct
  REGION 1..6: note = AC6-27 peptide selected for its ability to modulate theaggregation of the -amyloid peptide
TCSWFD

SEQ ID NO: 231 - protein, 6 aa, synthetic construct
  REGION 1..6: note = AC6-28 peptide selected for its ability to modulate theaggregation of the -amyloid peptide
TLEYFM

SEQ ID NO: 232 - protein, 6 aa, synthetic construct
  REGION 1..6: note = AC6-32 peptide selected for its ability to modulate theaggregation of the -amyloid peptide
TLCWLN

SEQ ID NO: 233 - protein, 6 aa, synthetic construct
  REGION 1..6: note = AC6-36 peptide selected for its ability to modulate theaggregation of the -amyloid peptide
TPIVFD

SEQ ID NO: 234 - protein, 6 aa, synthetic construct
  REGION 1..6: note = AC6-37 peptide selected for its ability to modulate theaggregation of the -amyloid peptide
TLWVFD

SEQ ID NO: 235 - protein, 6 aa, synthetic construct
  REGION 1..6: note = AC6-40 peptide selected for its ability to modulate theaggregation of the -amyloid peptide
TPLWFN

SEQ ID NO: 236 - protein, 6 aa, synthetic construct
  REGION 1..6: note = AC6-41 peptide selected for its ability to modulate theaggregation of the -amyloid peptide
TSVEYE

SEQ ID NO: 237 - protein, 6 aa, synthetic construct
  REGION 1..6: note = AC6-42 peptide selected for its ability to modulate theaggregation of the -amyloid peptide
TLGWLD

SEQ ID NO: 238 - protein, 6 aa, synthetic construct
  REGION 1..6: note = AC6-44 peptide selected for its ability to modulate theaggregation of the -amyloid peptide
TPPWFD

SEQ ID NO: 239 - protein, 6 aa, synthetic construct
  REGION 1..6: note = AC6-46 peptide selected for its ability to modulate theaggregation of the -amyloid peptide
TPCWFD

SEQ ID NO: 240 - protein, 6 aa, synthetic construct
  REGION 1..6: note = AC6-47 peptide selected for its ability to modulate theaggregation of the -amyloid peptide
TLSWYD

SEQ ID NO: 241 - protein, 6 aa, synthetic construct
  REGION 1..6: note = AC6-48 peptide selected for its ability to modulate theaggregation of the -amyloid peptide
TPVLVD

SEQ ID NO: 242 - protein, 6 aa, synthetic construct
  REGION 1..6: note = AC6-49 peptide selected for its ability to modulate theaggregation of the -amyloid peptide
TLEYLW

SEQ ID NO: 243 - protein, 6 aa, synthetic construct
  REGION 1..6: note = AC6-50 peptide selected for its ability to modulate theaggregation of the -amyloid peptide
TIFWFD

SEQ ID NO: 244 - protein, 6 aa, synthetic construct
  REGION 1..6: note = AC6-53 peptide selected for its ability to modulate theaggregation of the -amyloid peptide
TPALVD

SEQ ID NO: 245 - protein, 6 aa, synthetic construct
  REGION 1..6: note = AC6-55 peptide selected for its ability to modulate theaggregation of the -amyloid peptide
TPGWFD

SEQ ID NO: 246 - protein, 6 aa, synthetic construct
  REGION 1..6: note = AC6-57 peptide selected for its ability to modulate theaggregation of the -amyloid peptide
TLSVFD

SEQ ID NO: 247 - protein, 6 aa, synthetic construct
  REGION 1..6: note = AC6-58 peptide selected for its ability to modulate theaggregation of the -amyloid peptide
TPGLVD

SEQ ID NO: 248 - protein, 6 aa, synthetic construct
  REGION 1..6: note = AC6-59 peptide selected for its ability to modulate theaggregation of the -amyloid peptide
TLSWFN

SEQ ID NO: 249 - protein, 6 aa, synthetic construct
  REGION 1..6: note = AC6-63 peptide selected for its ability to modulate theaggregation of the -amyloid peptide
TLDFFD

SEQ ID NO: 250 - protein, 6 aa, synthetic construct
  REGION 1..6: note = AC6-65 peptide selected for its ability to modulate theaggregation of the -amyloid peptide
TPSWFD

SEQ ID NO: 251 - protein, 6 aa, synthetic construct
  REGION 1..6: note = AC6-68 peptide selected for its ability to modulate theaggregation of the -amyloid peptide
TPALFD

SEQ ID NO: 252 - protein, 6 aa, synthetic construct
  REGION 1..6: note = AC6-69 peptide selected for its ability to modulate theaggregation of the -amyloid peptide
TPAWSD

SEQ ID NO: 253 - protein, 6 aa, synthetic construct
  REGION 1..6: note = AC6-78 peptide selected for its ability to modulate theaggregation of the -amyloid peptide
TPARFD

SEQ ID NO: 254 - protein, 6 aa, synthetic construct
  REGION 1..6: note = AC6-79 peptide selected for its ability to modulate theaggregation of the -amyloid peptide
TPAWLD

SEQ ID NO: 255 - protein, 6 aa, synthetic construct
  REGION 1..6: note = AC6-80 peptide selected for its ability to modulate theaggregation of the -amyloid peptide
TPVWLD